European Patent Application EP 4 772 648 A1, published July 8, 2026. Title: 一种嘌呤核苷的制备方法. Applicant: 天津凯莱英生物科技有限公司. Application CN 202311820673.7, filed December 27, 2023. The sequence listing filed with the application follows.

SEQUENCE LISTING (6 sequences)

SEQ ID NO: 1 - protein, 440 aa, Escherichia coli
  source 1..440: note = TP
MFLAQEIIRKKRDGHALSDEEIRFFINGIRDNTISEGQIAALAMTIFFHDMTMPERVSLTMAMRDSGTVLDWKSLHLNGPIVDKHSTGGVGDVTSLMLGPMVAACGGYIPMISGRGLGHTGGTLDKLESIPGFDIFPDDNRFREIIKDVGVAIIGQTSSLAPADKRFYATRDITATVDSIPLITASILAKKLAEGLDALVMDVKVGSGAFMPTYELSEALAEAIVGVANGAGVRTTALLTDMNQVLASSAGNAVEVREAVQFLTGEYRNPRLFDVTMALCVEMLISGKLAKDDAEARAKLQAVLDNGKAAEVFGRMVAAQKGPTDFVENYAKYLPTAMLTKAVYADTEGFVSEMDTRALGMAVVAMGGGRRQASDTIDYSVGFTDMARLGDQVDGQRPLAVIHAKDENNWQEAAKAVKAAIKLADKAPESTPTVYRRISE

SEQ ID NO: 2 - protein, 433 aa, Geobacillus stearothermophilus
  source 1..433: note = PyNP
MRMVDLIEKKRDGHALTKEEIQFIIEGYTKGDIPDYQMSALAMAIFFRGMNEEETAELTMAMVHSGDTIDLSRIEGIKVDKHSTGGVGDTTTLVLGPLVASVGVPVAKMSGRGLGHTGGTIDKLESVPGFHVEITNDEFIDLVNKNKIAVVGQSGNLTPADKKLYALRDVTATVNSIPLIASSIMSKKIAAGADAIVLDVKTGVGAFMKDLNDAKALAKAMVDIGNRVGRKTMAIISDMSQPLGYAIGNALEVKEAIDTLKGEGPEDFQELCLVLGSHMVYLAEKASSLEEARHMLEKAMKDGSALQTFKTFLAAQGGDASVVDDPSKLPQAKYIIELEAKEDGYVSEIVADAVGTAAMWLGAGRATKESTIDLAVGLVLRKKVGDAVKKGESLVTIYSNREQVDDVKQKLYENIRISATPVQAPTLIYDKIS

SEQ ID NO: 3 - protein, 235 aa, Geobacillus thermoglucosidasius
  source 1..235: note = PNP
MSIHIEAKQQEIAEKILLPGDPLRAQYIAETFLEGATCYNRVRGMLGFTGTYKGHRISVQGTGMGVPSISIYVNELIQSYHVQTLIRVGTCGAIQKDVNVRDVILAMSASTDSNMNRLTFRGRDYAPTANFALLRTAYEVGAEKGLPLKVGSVFTADMFYNDEPDWETWARYGVLAVEMETAALYTLAAKFGRKALSVLTVSDHILTGEETTAQERQTTFNDMIEVALETAIRVE

SEQ ID NO: 4 - DNA, 1323 bp, synthetic construct
  source 1..1323: mol_type = other DNA; note; note (original language) = 编码TP的核苷酸序列
atgtttctggcgcaggaaattattcgcaagaaacgcgatggccatgcgctgagcgatgaagaaattcgctttttcattaacggcatccgcgataacaccattagcgaaggccagattgcggcgctggcgatgactattttctttcatgatatgaccatgccggaacgcgtgagcctgacgatggcgatgcgtgatagcggcaccgttctggattggaaaagcctgcatctgaacggcccgattgtggataaacatagcaccggcggcgtgggcgatgtgaccagcttaatgttaggcccgatggtggcggcgtgcggcggttatattccgatgattagcggtcgcggcctgggccataccggtggtaccttagataaactggaaagcattccgggctttgatatttttccggatgataaccgctttcgcgaaattattaaagacgtgggcgtggcgattattggccagaccagcagcctggcgccggcggataaacgtttttatgcgacccgcgatattaccgcgaccgtggatagcattccgctgattaccgcgagcattctggcgaaaaagctggcggaaggcctggatgcgctggtgatggatgtgaaagtgggcagcggcgcgtttatgccgacctatgaactgagcgaagcgctggcggaagcgattgtgggcgttgcgaatggcgcgggcgtacgtaccaccgcactgttaaccgatatgaaccaggtgctggcgagcagcgcgggcaatgcggttgaagttcgtgaagcggttcaatttctgaccggcgaatatcgcaacccgcgcctgtttgatgtgacgatggcgctgtgcgtggaaatgctgattagcggcaaactggcgaaagatgatgcggaagcgcgtgccaaactgcaggcggttttagataacggcaaagcggcggaagtgtttggccgcatggtggcggcacaaaaaggccctactgattttgtggaaaactatgcgaaatatctgccgaccgcgatgctgaccaaagcggtgtatgcggataccgaaggctttgtgagcgaaatggatacccgcgccctgggcatggcggttgttgcgatgggtggtggtcgtcgtcaagcgagcgataccattgattatagcgtgggctttaccgatatggcgcgtctgggcgatcaggtggatggccaacgtcctttagcggtgattcatgcgaaagatgaaaacaactggcaggaagcggcgaaagcggtgaaagcggcgattaaactggcggataaagcgccggaaagcaccccgaccgtttatcgccgtattagcgaataa

SEQ ID NO: 5 - DNA, 1302 bp, synthetic construct
  source 1..1302: mol_type = other DNA; note; note (original language) = 编码PyNP的核苷酸序列
atgcgcatggtggatctgattgaaaaaaaacgcgatggccatgcgctgaccaaagaagaaattcagtttattattgaaggctataccaaaggcgatattccggattatcagatgagcgcgctggcgatggcgattttttttcgcggcatgaacgaagaagaaaccgcggaactgacgatggcgatggtgcatagcggcgataccattgatctgagccgcattgaaggcattaaagtggataaacatagtaccggaggcgtaggtgataccaccacccttgtactgggcccgcttgtggctagtgtgggcgtgccggtggcgaaaatgagtggccgcggcctgggccataccggcggcaccattgataaactggaaagcgtgccgggctttcatgtggaaattaccaacgatgaatttattgatctggtgaacaaaaacaaaattgcggtggtgggtcagagcggcaacctgaccccggcggataaaaaactgtatgcgctgcgcgatgtgaccgcgaccgtgaacagcattccgctgattgcgagcagcattatgagcaaaaaaattgcggcgggcgcggatgcgattgtgctggatgtgaaaaccggcgtgggcgcgtttatgaaggatctgaacgatgcgaaagcgctggcgaaagcgatggtggatattggcaaccgcgtgggccgcaaaacgatggcgattattagcgatatgagtcagccgctgggctatgcgattggcaacgcgctggaagtgaaagaagcgattgataccctgaaaggcgaaggcccggaagattttcaagaactgtgcctcgtgctgggcagccacatggtgtatctggcggaaaaagcgagcagcctggaagaagcgcgccacatgctggaaaaagcgatgaaagatggcagcgcgctgcagacctttaaaacctttctggcggcgcaaggcggcgatgcgagcgtggtggatgatccgagcaaactgccgcaagcgaaatatattattgaactggaagcgaaagaagatggctatgtgagcgaaattgtggcggatgcggtgggcaccgcggcgatgtggctgggcgcgggccgcgcgaccaaagaaagcaccattgatctggcggtgggcctggtgctgcgcaaaaaagtgggcgatgcggtgaaaaaaggcgaaagcctggtgaccatttatagcaaccgcgaacaagtggatgatgtgaaacagaaactgtatgaaaacattcgcattagcgcgaccccggtgcaagcgccgaccctgatttatgataaaattagctaa

SEQ ID NO: 6 - DNA, 708 bp, synthetic construct
  source 1..708: mol_type = other DNA; note; note (original language) = 编码PNP的核苷酸序列
atgagcattcatattgaagcgaaacagcaggaaattgcggaaaagattctgctgccgggcgatccgttacgtgcgcaatatattgcggaaacctttctggaaggcgcgacctgctataaccgcgtgcgcggtatgctgggctttaccggtacctataaaggccatcgcattagcgtgcagggcaccggcatgggcgttccgtcaattagcatttatgtgaacgaactgattcagagctatcacgtgcagaccctgattcgcgtgggcacctgtggcgcaattcagaaagatgtgaacgtgcgcgatgtgattctggcgatgagcgcgagcaccgatagcaacatgaaccgcctgacctttcgcggccgtgattatgcgcctaccgcgaattttgcgctgctgcgcactgcgtatgaagtgggcgcggaaaaaggcctgccgctgaaagtgggcagcgtgtttaccgcggatatgttttataacgatgaaccggattgggaaacctgggcccgctatggcgttctggcggtggaaatggaaaccgcggcgttatataccctggcggcgaaatttggccgcaaagcgctgagcgtgctgaccgtgagcgatcatattctgaccggcgaagaaaccaccgcgcaggaacgccaaaccacctttaacgatatgattgaagtggcgctggaaaccgcgattcgcgtggaataa